European Patent Application EP 4 699 610 A1, published February 25, 2026. Title: Pharmaceutical composition for treatment of glioma. Applicant: SymBio Pharmaceuticals Limited. Application WO. The sequence listing filed with the application follows.

SEQUENCE LISTING (4 sequences)

SEQ ID NO: 1 - DNA, 19 bp, synthetic construct
  source 1..19: mol_type = other DNA
gcaatgagaggcaatcctg

SEQ ID NO: 2 - DNA, 19 bp, synthetic construct
  source 1..19: mol_type = other DNA
ccagaagccattccttcac

SEQ ID NO: 3 - DNA, 17 bp, synthetic construct
  source 1..17: mol_type = other DNA
ccactcctccacctttg

SEQ ID NO: 4 - DNA, 17 bp, synthetic construct
  source 1..17: mol_type = other DNA
caccaccctgttgctgt